European Patent Application EP 4 806 918 A1, published September 16, 2026. Title: 靶向人源PD-L1的全人源抗体. Applicant: 南京蓬勃生物科技有限公司. Application CN 202311466254.8, filed November 6, 2023. The sequence listing filed with the application follows.

SEQUENCE LISTING (18 sequences)

SEQ ID NO: 1 - protein, 8 aa, synthetic construct
GRTALTYA

SEQ ID NO: 2 - protein, 8 aa, unidentified
INWSGSMT

SEQ ID NO: 3 - protein, 18 aa, synthetic construct
AATRTAITMPPQRDGVDY

SEQ ID NO: 4 - protein, 6 aa, synthetic construct
QDISNY

SEQ ID NO: 5 - protein, 9 aa, synthetic construct
QQYDNLPRT

SEQ ID NO: 6 - protein, 125 aa, synthetic construct
QVQLVDSGGGLVQAGGSLSVSCAVSGRTALTYAVGWFRQAPGKERDFVAGINWSGSMTNYADSVKGRFTISRDNQKNTVYLQMNSLKPEDTAVYYCAATRTAITMPPQRDGVDYWGKGTTVTVSS

SEQ ID NO: 7 - protein, 107 aa, synthetic construct
VIWMTQSPSSLSASVGDRVTITCQASQDISNYLNWYQQKPGKAPKLLIYDASNLETGVPSRFSGSGSGTDFTFTISSLQPEDIATYYCQQYDNLPRTFGQGTKVEIK

SEQ ID NO: 8 - protein, 8 aa, synthetic construct
GSSFSLAV

SEQ ID NO: 9 - protein, 7 aa, synthetic construct
ISSAAGT

SEQ ID NO: 10 - protein, 12 aa, synthetic construct
WRGAVPGDPYGR

SEQ ID NO: 11 - protein, 7 aa, synthetic construct
QSVSNNY

SEQ ID NO: 12 - protein, 9 aa, synthetic construct
QQYGNSPGT

SEQ ID NO: 13 - protein, 118 aa, synthetic construct
EVQLVQSGGGLVQPGGSLRLSCAGSGSSFSLAVMGWYRQAPGRQRELVGIISSAAGTNYADSVKGRFTISRDDAKNTLYLQMNSLTAEDTAVYYCWRGAVPGDPYGRWGQGTTVTVSS

SEQ ID NO: 14 - protein, 108 aa, synthetic construct
EIVMTQSPGTLSLSPGEGATLSCRASQSVSNNYLAWYQQKHGQAPRLLIYGASSRATGIPDRFSGSGSGTDFTLTINRLEPEDFALYYCQQYGNSPGTFGQGTKVDIK

SEQ ID NO: 15 - protein, 11 aa, synthetic construct
QSLVHSDGNTY

SEQ ID NO: 16 - protein, 9 aa, synthetic construct
MQGTHWPWT

SEQ ID NO: 17 - protein, 118 aa, synthetic construct
QVQLVQSGGGLVQPGGSLRLSCAGSGSSFSLAVMGWYRQAPGRQRELVGIISSAAGTNYADSVKGRFTISRDDAKNTLYLQMNSLTAEDTAVYYCWRGAVPGDPYGRWGQGTLVTVSS

SEQ ID NO: 18 - protein, 112 aa, synthetic construct
EIVLTQSPLSLPVTLGQPASISCRSSQSLVHSDGNTYLNWFQQRPGQPPRRLIYEVSNRDSGVPDRFSGSGSGTDFTLKISRVEAEDVGVYYCMQGTHWPWTFGQGTKVEIK